European Patent Application EP 4 524 247 A2, published March 19, 2025. Title: CRISPR/CAS9-MEDIATED EXON-SKIPPING APPROACH FOR USH2A-ASSOCIATED USHER SYNDROME. Applicant: MASSACHUSETTS EYE AND EAR INFIRMARY. Application EP. The sequence listing filed with the application follows.

SEQUENCE LISTING (189 sequences)

SEQ ID NO: 1 - DNA, 18241 bp, synthetic construct
  misc_feature 1..18241: note = Description of Artificial Sequence: Synthetic polynucleotide
  source 1..18241: mol_type = other DNA
tgtttgctctgcagaatactttacctgggcacccaagtcttccttccagcattcctgctgctacagcctatttgctgagtaaccaggggttacagcagcgttgccaggcaacgagggacagcggtcctgttgaagagccatttgtcacactgaggggactggttgaaatgcaataaagaaatgataccagcagctactcatgtcttcgccattgctaagaacgtcgttggtattaccttactctgagaacgtgtctgcagtttccagaaaatggagtatcgcaacatcacttaaagtaccctgcttcaaagtattgctggcaagtggcgtgggcctgattatttatttagaaatgctttatcaggaggagaatgcttttttgtaaacatgaattgcccagttctttcattgggctctggcttcttgtttcaggtcattgaaatgttgatctttgcctattttgcttcaatatccttgactgagtcacgaggtcttttcccaaggctggagaacgtgggagctttcaagaaagtttccatcgtgccaacccaagcagtatgtggactcccagaccgaagcactttttgtcacagctctgctgctgctgaaagtattcagttctgtacccagcggttttgtattcaggattgcccatacagatcttcacaccctacctacactgcccttttctcagcaggcctcagtagctgcatcacaccagacaagaatgatctgcatcctaacgcccatagcaattctgcaagttttatttttggaaatcacaagagctgcttttcttctcctccttctccaaagctgatggcatcatttaccttagctgtatggctgaaacctgagcaacaaggtgtaatgtgtgttatagaaaagacagtagatgggcagattgtgttcaaacttacaatatctgagaaagagaccatgttttattatcgcacagtaaatggtttgcaacctccaataaaagtaatgacactggggagaattcttgtgaagaaatggattcatcttagtgtgcaggtgcatcagacaaaaatcagcttctttatcaatggcgtggagaaggatcatacacctttcaatgcaagaactctaagtggttcaattacagattttgcatctggtactgtgcaaataggacagagtttaaatggtttagagcagtttgtcggaagaatgcaagattttcgattataccaagtggcacttacaaacagagagattctggaagtcttctctggagatcttctcagattgcatgcccaatcacattgccgttgccctggcagccacccgcgggtccaccctttggcacagcggtactgcattcctaatgatgcaggagacacagctgataatagagtgtcacggttgaatcctgaagcccatcctctctcttttgtcaatgataatgatgttggtacttcatgggtttcaaatgtgtttacaaacattacacagcttaatcaaggagtgactatttcagttgatttggaaaatggacagtatcaggtgttttatattatcattcagttctttagtccacaaccaacggaaataaggattcaaaggaagaaggaaaatagtttagattgggaggactggcaatattttgccaggaattgtggtgcttttggaatgaaaaacaatggagatttggaaaaacctgattctgtcaactgtcttcagctttccaattttactccatattcccgtggcaatgtcacatttagcatcctgacacctggaccaaattatcgtcctggatacaataacttctataataccccatctcttcaagagttcgtaaaagccacgcaaataaggtttcattttcatgggcagtactatacaactgagactgctgttaacctcagacacagatattatgcagtggacgaaatcaccattagtgggagatgtcagtgccatggtcatgccgataactgcgacacaacaagccagccatatagatgcctctgctcccaggagagcttcactgaaggacttcattgtgatcgctgcttgcctctttataatgacaagcctttccgccaaggtgatcaagtttacgctttcaattgtaaaccttgtcaatgcaacagccattccaaaagctgccattacaacatctctgtagacccatttccttttgagcacttcagagggggaggaggagtttgtgatgattgtgagcataacactacaggaaggaactgtgagctgtgcaaggattactttttccgacaagttggtgcagatccttcggccatagatgtttgcaaaccctgtgactgtgatacagttggcactagaaatggtagcattctttgtgatcagattggaggacagtgtaattgtaagagacacgtgtctggcaggcagtgcaatcagtgccagaatggattctacaatctacaagagttggatcctgatggctgcagtccctgtaactgcaatacctctgggacagtggatggagatattacctgtcaccaaaattcaggccagtgcaagtgcaaagcaaacgttattggtttttatatttctccaggcaatgccactggctgcctgccatgctcatgccatacaactggtgcagttaatcacatctgtaatagcctgactggtcagtgtgtttgccaagatgcttccattgctgggcaacgttgtgaccaatgcaaagaccattactttggatttgatcctcagactggaagatgtcagccttgtaattgtcatctctcaggagccttgaatgaaacctgtcacttggtcacaggccagtgtttctgtaaacaatttgtcactggctcaaagtgtgatgcttgtgttcccagtgcaagccacttggatgtcaacaatctattgggttgcagcaaaactccattccagcaacctccgcccagaggacaagttcaaagttcttctgctatcaatctctcctggagtccacctgattctccaaatgcccactggcttacttacagtttactcagggatggttttgaaatctacacaacagaggatcaatacccatacagtattcaatacttcttagacacagacctgttaccatataccaaatattcctattacattgagaccaccaatgtgcatggttcaacaaggagtgtagctgtcacttacaagacaaaaccaggggtcccagagggaaacttgactttaagttatatcattcctattggctcagactctgtgacacttacctggacaacactctcaaatcaatctggtcccatagagaaatatattttgtcctgtgcccctttggctggtggtcagccatgtgtttcctacgaaggtcatgaaacctcagctaccatctggaatctggttccatttgccaagtacgatttttctgtacaggcgtgtactagcgggggctgtttacacagcttgcccattacagtgaccacagcccaggcccctccccaaagactaagtccacctaagatgcagaaaatcagttctacagaacttcatgtagaatggtctccaccagcggaactaaatggaataattataagatatgaactatacatgagaagactgagatctactaaagaaaccacatctgaggaaagtcgagtttttcagagcagtggttggctcagtcctcattcatttgtagaatcggccaatgaaaatgcattaaaacctcctcaaacaatgacaaccatcactggcttggagccatacaccaagtatgagttcagagtcttagctgtgaatatggctggaagtgtgtcttctgcctgggtctcagaaagaacgggagaatcagcacctgtattcatgatccctccttcagtctttcccctctcttcgtactctctcaatatctcctgggagaagccagcagataatgttacaagaggaaaagttgtggggtatgacatcaatatgctttctgaacaatcacctcaacagtctattcccatggcgttttcacagctgttgcacactgctaaatcccaagaactatcttacactgtagaaggactgaaaccttataggatatatgagtttactattactctctgcaattcagttggttgtgtgaccagtgcttcgggagcaggacaaactttagcagcagcaccagcacaactgaggccacctctggttaaaggaatcaacagcacaacaatccatcttaagtggtttccacctgaagaactgaatggaccctctcctatatatcagctggaaaggagagagtcatctctaccagctctgatgaccacgatgatgaaaggaatccgtttcataggaaatgggtattgtaaatttcccagctccactcacccagtcaatacagacttcactggcattaaggccagctttcgaacaaaagtgcctgaaggtttgattgtctttgcagcatcacctggcaatcaggaagagtattttgcacttcagttgaagaagggacgtctttattttctttttgatcctcaggggtcaccagtggaagtaactacaactaatgatcatggcaaacaatatagtgatggaaaatggcatgaaataattgctattaggcatcaggcttttggccaaatcactctggatgggatatatacaggttcctctgccatcctgaatggtagtactgttattggagataacacaggagtctttctgggagggctcccgcgaagttataccatcctcaggaaggatcctgagataatccaaaaaggttttgtgggctgtctcaaggatgtacattttatgaagaattacaatccgtcagctatttgggaacctctggattggcagagttctgaagaacaaatcaacgtgtataacagctgggagggatgtcccgcttcattaaatgagggagctcagttcctaggagcagggttcctggaacttcatccatatatgtttcatggtggaatgaactttgagatttcctttaagttcagaactgaccaattaaatggattgcttcttttcgtttataacaaagatggacctgattttcttgctatggagctgaaaagtggaatattgaccttccggttaaataccagtcttgcctttacacaagtggatctattgctggggctatcctattgtaatggaaagtggaataaagtcattattaaaaaggaaggctctttcatatcagcaagtgtgaatggactgatgaagcatgcatcggagtccggagaccagccactggtggtgaattcaccagtttatgtgggaggaatcccacaggaactgctgaactcttatcaacatttgtgtttggaacaaggtttcggtggttgcatgaaggatgttaaatttacacggggtgctgtcgttaacttggcatctgtgtccagcggtgctgtcagagtcaatctggatggatgcctatcaactgacagtgctgttaactgcaggggaaatgactccatcctggtttaccagggaaaagagcagagtgtttacgagggtggtctccagccttttacagaatacctgtatcgagtgatagcctcgcatgaaggaggttcagtatatagtgattggagtcgaggacgtacaacaggagcagctccacaaagtgtgccaactccctcaagagtccgcagcttaaatggatacagcattgaggtgacctgggatgaacctgttgtcagaggtgtaattgagaagtacattctgaaagcctatagtgaggacagcacccgtccaccccgcatgccctctgccagtgctgaatttgtcaatacaagcaacctcacaggcatattgacaggcttgctacccttcaaaaactatgcagtaaccctaactgcttgcactttggctggctgtactgagagctcacatgcattgaacatctctactccacaagaagccccacaagaggttcagccaccagtagccaaatcccttcccagttctttgctgctctcctggaacccacccaaaaaggcaaatggtattataactcagtactgtttatacatggatgggaggctgatctattcaggcagtgaggagaactacacagtcacagatttagcagtatttacaccccaccagtttctactaagtgcatgcacacatgtgggctgtacaaacagttcctgggtcctactgtacacagcacagctgccaccagaacacgtggattccccagttctgactgtcctggattctagaactatacacatacagtggaaacaaccaagaaaaataagtgggattctggaacgctatgtattatatatgtcaaaccatacacatgattttacaatttggagtgtcatctataacagtacagaacttttccaggatcatatgctacaatacgttttacctggtaataaatatctcatcaagctgggagcttgcacaggtggtgggtgcacagtgagtgaggccagtgaggccctaactgacgaggacatacccgaaggcgtgccagcccccaaagcccactcatattcacctgactcctttaatgtctcctggactgagcctgaatatccgaatggtgttatcacgagttatggattatatctagatggtatattaatccacaattcctcagaactcagctatcgtgcttacggatttgctccttggagtttacattccttcagagtccaagcatgcacggccaaaggttgtgctctgggcccactggtggaaaatcgaactctagaagctcctcctgaaggaacagtaaatgtgtttgtcaaaacacagggatcccggaaagcccacgtgaggtgggaagcaccttttcgccctaatggactcttaacacactcagtccttttcactgggatattctatgtagacccagtaggtaataactacacccttctgaatgtcacaaaagtcatgtacagcggagaagagacaaacctttgggtgctcatcgatgggctggttccttttaccaactatactgtacaagtgaatatttcaaatagccaaggcagcttgataactgatcctataacaattgcaatgcctccaggagctccagatggcgtgctgcctcccaggctttcatctgccactccaaccagtcttcaggttgtctggtctacaccagctcgtaataacgctcctggctctcccagataccaactccagatgaggtctggcgactccacccatggatttctagagttattttccaatccttctgcatcgttaagctatgaagtgagtgatctccaaccgtacacagagtatatgtttcggttggttgcctccaatggatttggcagtgcacatagttcttggattccattcatgaccgcagaggacaaacctggacctgtagttcctccgattcttctggatgtgaagtcaagaatgatgttggtcacctggcagcatcctagaaaatccaatggggttattacccattataacatttatctacatggccgtctatacttgagaactcctggaaatgtcactaattgcacagtgatgcatttacacccatacactgcctataagtttcaggtagaagcctgcacttcaaaaggatgttccctttcaccagagtcccagactgtatggacactcccaggggcaccggaagggatcccaagtccagagctgttctctgatactccaacatctgtgattatatcttggcaaccccctacccaccccaatggcttggtggagaatttcacaattgagagaagagtcaaaggaaaggaagaagttactaccctggtgactctcccgaggagtcattccatgaggtttattgacaagacttctgctcttagcccatggacaaaatatgaatatcgggtactgatgagcactcttcatggaggcacaaacagcagtgcttgggtagaagttaccacaagaccctcacgacctgctggggtgcagccacctgtggtgacagtgctggaacccgatgcagtccaggtcacttggaaacccccactcatccagaacggagacatacttagctatgagattcacatgcctgaccctcacatcactttaaccaatgtgacttccgcagtgttaagtcaaaaagttactcatctgattcctttcactaattattctgtcaccattgttgcttgctcagggggtaatgggtaccttggagggtgcacagagagtttacctacctatgttaccactcaccccaccgtacctcagaatgttggcccattgtctgtgattccactaagtgaatcatatgttgtgatttcttggcaaccaccatccaagccaaatggacctaatttgagatatgagcttctgagacgtaaaatccagcagccacttgcatcaaatcccccagaagatttaaatcggtggcacaatatttattcaggaactcagtggctttatgaagataagggtcttagcaggtttacaacctatgaatatatgctcttcgtacacaacagtgtgggttttacaccgagccgagaagtgactgtgacaacgttagctggtcttccagagagaggagccaatctcactgcgagtgtccttaaccacacagccatcgacgtgaggtgggctaaaccaactgttcaagacctacaaggtgaagttgaatattacacacttttttggagttctgctacctcaaacgactctctaaaaatcttgccagatgtaaactctcatgtcattggccacctaaagccaaacacagagtattggatctttatctctgtcttcaatggagtccacagcatcaacagtgcaggacttcatgcaaccacttgcgatggggagcctcagggcatgcttcctccagaggttgtcatcatcaacagtacagctgtacgtgtcatctggacatctccttcaaacccaaatggtgttgtcactgagtattctatctatgtaaataataagctctacaagactggaatgaatgtgcctgggtcgtttattctgagagacctgtctcccttcactatctatgacattcaggttgaagtctgcacaatatatgcctgcgtgaaaagcaatggaacccaaattaccactgtggaagacactccaagtgatataccaacacccacaattcgtggcatcacttcaagatctcttcaaattgattgggtgtctccacggaagccaaatggcatcattcttggatatgatctcctatggaaaacatggtatccatgcgctaaaactcaaaagttagtgcaggatcagagtgatgagctctgcaaggcagtgaggtgtcaaaaacctgaatctatctgtggacacatttgctattcttctgaagctaaggtttgttgtaacggagtgctctataaccccaagcctggacatcgctgttgtgaagaaaagtatatcccgtttgttctgaattctactggagtttgttgtggtggccgaatacaggaggcacaaccaaatcatcagtgctgctctgggtattacgctagaattctaccaggtgaagtatgctgtccagatgaacagcacaatcgggtttctgttggcattggtgattcctgctgtggcagaatgccgtactccacctcaggaaaccagatttgctgtgctgggaggcttcatgatggccatggccagaagtgctgtggcagacagattgtgagcaacgatttagagtgttgtggtggagaagaaggagtggtgtacaatcgccttccaggtatgttctgttgtgggcaggattatgtgaatatgtcagataccatatgctgctcagcttccagtggagagtctaaagcacatattaaaaagaatgacccggtgccagtaaaatgctgtgagactgaacttattccaaagagccagaaatgctgtaatggagttggatataatcctttgaaatatgtttgctctgacaagatttcaactggaatgatgatgaaggaaaccaaagagtgcaggatcctctgcccagcatctatggaagccacagaacattgtggcaggtgtgacttcaactttaccagccacatttgcactgtgataagagggtctcacaattccacagggaaggcatcaattgaagaaatgtgttcatctgccgaagaaaccattcatacagggagtgtaaacacgtactcttacacagatgtgaacctcaagccctacatgacatatgagtacaggatttctgcctggaacagctatgggcgaggactcagcaaagctgtgagagccagaacaaaagaagatgtgcctcaaggagtgagtccccctacgtggaccaaaatagacaatcttgaagatacaattgtcttaaactggagaaaacctatacaatcaaatggtcctattatttactacatccttcttcgaaatggaattgaacgttttcggggaacatcactgagcttctctgataaagagggaattcaaccatttcaggaatattcatatcagctgaaagcttgcacggttgctggctgtgccaccagtagcaaggtagttgcagctactacccaaggagttccggagagcatcctgccaccaagcatcacagccctaagtgcagtggctctgcatctgagctggagtgtccctgagaaatcaaacggcgtcattaaagagtaccagatcaggcaggttgggaaaggtctcatccacactgacaccactgacaggagacagcatacggtcacaggtctccagccatacaccaactacagcttcactcttacagcttgtacatctgctgggtgcacttcaagcgagccttttctaggtcagacactgcaggcagctcctgaaggagtttgggtgacacctcgacacattatcatcaattctacaacagtggaattatattggagtctgccagaaaagcccaatggcctcgtttctcaatatcaattgagtcgtaatggaaacttgcttttcctgggtggcagtgaggagcagaatttcactgataaaaacctggagcccaatagcagatacacttacaagttagaagtcaaaactggaggtggcagcagtgctagtgatgattacattgttcaaacacctatgtcaacaccagaagaaatctatcctccatataatatcacagtaattgggccttattctatatttgtagcttggataccaccagggatcctcatccccgaaattcctgtggagtacaatgtcttactcaatgatggaagtgtaacacctctggccttctccgttggtcatcatcaatccacccttctggaaaatttgactccattcacacagtatgagataaggatacaagcatgtcaaaatggaagttgtggagttagcagtaggatgtttgtcaaaacacctgaagcagccccaatggatcttaattctcctgttcttaaggcactggggtcagcttgcatagagattaagtggatgccacctgaaaaaccaaatggaatcatcatcaactactttatttacagacgccctgctggcattgaagaggagtctgttttatttgtctggtcagaaggagcccttgaatttatggatgaaggagacaccctgaggcctttcacactctacgaatatcgggtcagagcctgtaactccaagggttcagtggagagtctgtggtcattaacacaaactctggaagctccacctcaagattttccagctccttgggctcaagccacgagtgctcattcagttctgttgaattggacaaagccagaatctcccaatggcattatctcccattaccgtgtggtctaccaggagagacccgacgatcctacatttaacagccctaccgtgcatgctttcacagtgaagggaacaagccatcaagcccacctgtacgggttagaaccattcacaacatatcgcattggtgttgtggctgcaaaccatgcaggagaaattttaagcccttggactctgattcaaaccttagaatcttccccaagtggactgagaaactttatagtagaacagaaagagaatggccgggcattgctactacagtggtcagaacctatgagaaccaatggtgtgattaagacatacaacatcttcagtgacgggttcctggagtactctggtttgaatcgtcagtttctcttccgccgcctggatcctttcactctctacacactgaccctggaggcctgcaccagagcaggttgtgcacactcggcgcctcagcctctgtggacagatgaagcccctccagactctcagctggctcctactgtccactctgtgaagtccaccagtgttgagctgagctggtctgagcctgttaacccaaatggaaaaataattcgctatgaagtgattcgcagatgcttcgagggaaaagcttggggaaatcagacgatccaggccgacgagaaaattgttttcacagaatataacactgaaaggaatacatttatgtataatgacacaggtttgcaaccatggacgcagtgtgaatataaaatctacacttggaattcagctgggcatacctgtagctcttggaatgtggtgaggacattgcaagcacctccagaaggtctctctccacctgtgatatcctatgtttctatgaatccccaaaaactgctgatttcctggatcccaccagaacagtctaatggtattatccagtcctataggcttcaaaggaatgaaatgctctatccttttagctttgatcctgtgactttcaattacactgatgaagagcttcttcctttttccacctatagctatgcactccaagcctgcacgagtggaggatgctccaccagcaaacccaccagcatcacaactctggaggctgctccatcagaagtcagccctccagatctttgggccgtcagtgccactcaaatgaatgtatgttggtcaccgcccacagtgcaaaatggaaagattactaaatatttagttagatatgataataaagagtcccttgctggccagggcctgtgcctgctggtttcccacctgcagccttactctcagtataacttctcccttgtagcctgcacgaatggaggttgcacagctagtgtgtcaaaatctgcctggacaatggaggccctgccagagaacatggactctccaacattgcaagtcacaggctcagaatcaatagaaatcacctggaaacctccaagaaacccaaatggccagatcagaagttatgaacttaggagggatggaaccattgtatatacaggcttggaaacacgctatcgtgattttactctcaccccaggtgtggagtatagctacacagtaactgccagcaacagccaagggggtattttgagtcctcttgtcaaagatcgaaccagcccctcagcaccctcagggatggaacctccaaaattgcaggccaggggtcctcaggagatcttagtgaactgggaccctccagtgagaacaaatggtgatatcatcaattataccctcttcatccgtgaactatttgaaagagaaactaaaatcatacacataaacacaactcataattcttttggtatgcagtcatatatagtaaaccagctgaagccatttcacaggtatgaaatacgaattcaagcgtgcaccaccctgggatgtgcatcaagtgactggacattcatacagacccctgagattgcacctttgatgcaaccccctccacatctggaggtacaaatggctccaggaggattccagccaactgtttctcttttgtggacaggaccgctgcagccaaatggaaaagttttgtattacgaattatacagaagacaaatagcaactcagcctagaaaatccaatccagtcctaatctataacggaagctcaacatcttttatagattccgaactattgcctttcacagagtatgagtatcaggtctgggcagtgaattctgcaggaaaagcccccagtagctggacatggtgcagaaccgggccagccccaccagaaggtctcagagcccccacgttccatgtgatctcttctacccaagcagtggtcaacatcagtgcccctgggaagcccaacgggatcgtcagtctctacaggctgttctccagcagcgcccatggggctgagacagtgctatccgaaggcatggccacccagcagactctccatggccttcaagccttcactaactactctattggagtagaggcctgcacctgcttcaactgttgcagcaaaggaccgacagctgaactgagaacccatcctgccccaccctcaggactgtcctctccacaaatcgggacgctggcctcaaggacggcctccttccggtggagtccccccatgttccccaatggtgtcattcacagctatgaactccaattccacgtggcttgccctcctgactcagccctcccctgtactcccagccaaatagaaacaaagtacacggggctggggcagaaagccagccttgggggtctccagccctacaccacatacaagctgagagtggtggcacacaacgaggtgggcagtacggcttccgagtggatcagtttcaccacccaaaaagaattgcctcagtaccgagccccattttcggtggacagcaatttgtctgtggtgtgtgtgaactggagtgacaccttcctcctgaacggccaactgaaggagtacgtgttaaccgacggagggcgacgcgtgtacagcggcttggacaccaccctctacataccgagaacggcggacaaaaccttctttttccaggtcatctgcacgactgacgaaggaagtgttaagacgccgttgatccaatatgatacctctactggacttggcttggtcctaacaactcctgggaaaaagaagggatcgcggagcaaaagcacagagttctacagcgagctgtggttcatagtgttaatggcgatgctgggcttgatcttgttggccatttttctgtccctgatactacaaagaaaaatccacaaagagccatatatcagagaaagacctcccttggtacctcttcagaagaggatgtctccattgaatgtttacccaccgggggaaaaccatatggggttagccgataccaaaattccccggtctgggacacctgtgagtatccgcagcaaccggagtgcatgtgtcctgcgcatcccgagtcaaaaccaaaccagcctaacctactcccagggttctcttcaccgcagcgtcagccagctcatggacattcaagacaagaaagtcttgatggacaactcactgtgggaagccatcatgggccacaacagtggactgtatgtggatgaagaggacctgatgaacgccatcaaggatttcagctcagtgactaaggaacgcaccacattcacagacacccacctgtaaaggatggaaacccagaagacgtaaccctggaatgcaaggtctgcacccatttcctcctgggttatcactcacacatcataaatgctgaaaagccattgtttattatcctataattctttaaagaaatgatgactgtttttgaaagtgttccttcctaatagaggtctaagaaatgatatttttctcatcttaaatgagagagaatattcatatgaaaatacttgatttgctcttattttgtagaagacaaagaagtatgtaattgtcacttggttctgtttggcagtgatgctcctggttaactgaataatcagtggcaatttcaagatggctcacagttgttagaagtagtaagttagttactggctcaaaaatgattctgttgaaaggatgtcactgctgttcatttctatctgccatttctgtcagggttgacacaatcctgcaagaatagttattctaatgatcacagctgctaaatgaatcccaaactttgcaccaggtcgacaaacttttctgaaggttctatttatttaccatacatagggttacttaccaaactttttgacaaggctgaaggttctatttatttacaatacatagggttactcaccaaactttttgacaaggcaacacataacttacacataaatgtctctgttcttgcatttatgaattttccaaaaatctaaggagtaaacagcttatttatacattttgaggagaaaacaaagtgtttcactaggaacacctctacttgaaccaatgtttttatttcatatattttatagttttgaaactagtttctcataaaattctgtcaattcactgaatatcagagaatactgacatcttcaacctagcacatttcaaatggaaactactgttctatttgcaatattaggctgcgtgaaattttaaaaggaaaaatgtatctgttccttctagcattaacatatatacatgtagagacaagactatacctatgtgtatatatatgtatatcatgtatatattactctgcactatatcccttctttttggagaactagccattattttagccacagaatcagtaagaacagatgatatgcaacagtaccaattacggttcaaaaatgtctgtcacctgctctagttggattacaaagtcattggtgaaagtcctatggcaagaaaaattttcttgcaaatcatccacataaaatcagatatttaaatttgttcttcatggaaaacagagtaagaaaacctcttgtcttccttcatccttaaaggtctttgtgaccccaggaaaatattgactctgtctaacacacaatagtcacaatactttttgtgaatctacaaccagagacaggcaaaaacttgtaaagtaagggatagtcttacttattctgcctgaaaacaatgtattaccccagggcccaacagtaaaagattgtggactttttgggtattgagatttcatctagctctgtgagagagcagctcctcagactgaccaactcctagacaaagtttgccaaccataagtgtcaaaagcacaggccagtattaagcagaagttctaccaccttattagaactgctataaacaaaagcatctgaaataattgtgcacatctggcagtgactgtagaaaatacgaaatatatatttctcgccaagtttttatactttctgaaatgaaaacataggattgactagtttactggtttttattcccatatgccgattctgggacaataaagttgtttaaagctggcacaaataagcattaaccaaggctgtgtccaccttctgtgagctacttaaggtatataggaaaggagtggtcacaaacttgcatcctaatccttggtggactcttctaagaatacagtttgctagtcacaaagaatagtctacaaatatgctttgctaggttcagaagattgagtttatcctgatttttgaaaaattaaccaggtatctttatcactgtgtatttttccaagcacagtataaaattttaacaacgcacaaaaaaatacagaactgcaggggattttatcttggatcattatccatttaatcatctaattagacatgaactcagttagctgaatcatttacattttgactccatagcttagggcagacagaagcctgtatggcttctgcccagaactctgtcccctgctacatgtctaagtttacttgtatttatttcagagaagaactctaagatgttgctttgctactttaagtggtattgcgtgccaagcctctattatacaaaccatgcagactcgcctctagagattctgattcggttgatctggggtgtgtggctgaggcatcagtactttttaaagcttccaggtgttctaatgttgagacccactgatgttccacaatctggaagaaatcatgtacaggaataatatgctatgcacagggactatgctccttggctcaccccttctcccttataaacaatgagcagttcttgatgaacctctttaaatttaaatctcctgactcacattttaccaattgtacatgccacattctcagcttacgaactaccatgttttgttattcttaatatcaactgtttggtaagagtacagttgtttttatacactctaagaaatgtgtttataatctactgtaatttccactaaatggaacccaaatattaatgttatggtaccatatactgatgtaaaaatcatgctggcatccatgaacacaccggtaaataaaacatagtccaagtggaagaattcattaataaggaacttttaattatgtcacaaatgaatagttggtttccaatgcacaaatatcatgtaaactaatctaaagatggtttgcttaataaatatttgaatgtgacc

SEQ ID NO: 2 - protein, 4988 aa, synthetic construct
  REGION 1..4988: note = Description of Artificial Sequence: Synthetic polypeptide
MNCPVLSLGSGFLFQVIEMLIFAYFASISLTESRGLFPRLENVGAFKKVSIVPTQAVCGLPDRSTFCHSSAAAESIQFCTQRFCIQDCPYRSSHPTYTALFSAGLSSCITPDKNDLHPNAHSNSASFIFGNHKSCFSSPPSPKLMASFTLAVWLKPEQQGVMCVIEKTVDGQIVFKLTISEKETMFYYRTVNGLQPPIKVMTLGRILVKKWIHLSVQVHQTKISFFINGVEKDHTPFNARTLSGSITDFASGTVQIGQSLNGLEQFVGRMQDFRLYQVALTNREILEVFSGDLLRLHAQSHCRCPGSHPRVHPLAQRYCIPNDAGDTADNRVSRLNPEAHPLSFVNDNDVGTSWVSNVFTNITQLNQGVTISVDLENGQYQVFYIIIQFFSPQPTEIRIQRKKENSLDWEDWQYFARNCGAFGMKNNGDLEKPDSVNCLQLSNFTPYSRGNVTFSILTPGPNYRPGYNNFYNTPSLQEFVKATQIRFHFHGQYYTTETAVNLRHRYYAVDEITISGRCQCHGHADNCDTTSQPYRCLCSQESFTEGLHCDRCLPLYNDKPFRQGDQVYAFNCKPCQCNSHSKSCHYNISVDPFPFEHFRGGGGVCDDCEHNTTGRNCELCKDYFFRQVGADPSAIDVCKPCDCDTVGTRNGSILCDQIGGQCNCKRHVSGRQCNQCQNGFYNLQELDPDGCSPCNCNTSGTVDGDITCHQNSGQCKCKANVIGFYISPGNATGCLPCSCHTTGAVNHICNSLTGQCVCQDASIAGQRCDQCKDHYFGFDPQTGRCQPCNCHLSGALNETCHLVTGQCFCKQFVTGSKCDACVPSASHLDVNNLLGCSKTPFQQPPPRGQVQSSSAINLSWSPPDSPNAHWLTYSLLRDGFEIYTTEDQYPYSIQYFLDTDLLPYTKYSYYIETTNVHGSTRSVAVTYKTKPGVPEGNLTLSYIIPIGSDSVTLTWTTLSNQSGPIEKYILSCAPLAGGQPCVSYEGHETSATIWNLVPFAKYDFSVQACTSGGCLHSLPITVTTAQAPPQRLSPPKMQKISSTELHVEWSPPAELNGIIIRYELYMRRLRSTKETTSEESRVFQSSGWLSPHSFVESANENALKPPQTMTTITGLEPYTKYEFRVLAVNMAGSVSSAWVSERTGESAPVFMIPPSVFPLSSYSLNISWEKPADNVTRGKVVGYDINMLSEQSPQQSIPMAFSQLLHTAKSQELSYTVEGLKPYRIYEFTITLCNSVGCVTSASGAGQTLAAAPAQLRPPLVKGINSTTIHLKWFPPEELNGPSPIYQLERRESSLPALMTTMMKGIRFIGNGYCKFPSSTHPVNTDFTGIKASFRTKVPEGLIVFAASPGNQEEYFALQLKKGRLYFLFDPQGSPVEVTTTNDHGKQYSDGKWHEIIAIRHQAFGQITLDGIYTGSSAILNGSTVIGDNTGVFLGGLPRSYTILRKDPEIIQKGFVGCLKDVHFMKNYNPSAIWEPLDWQSSEEQINVYNSWEGCPASLNEGAQFLGAGFLELHPYMFHGGMNFEISFKFRTDQLNGLLLFVYNKDGPDFLAMELKSGILTFRLNTSLAFTQVDLLLGLSYCNGKWNKVIIKKEGSFISASVNGLMKHASESGDQPLVVNSPVYVGGIPQELLNSYQHLCLEQGFGGCMKDVKFTRGAVVNLASVSSGAVRVNLDGCLSTDSAVNCRGNDSILVYQGKEQSVYEGGLQPFTEYLYRVIASHEGGSVYSDWSRGRTTGAAPQSVPTPSRVRSLNGYSIEVTWDEPVVRGVIEKYILKAYSEDSTRPPRMPSASAEFVNTSNLTGILTGLLPFKNYAVTLTACTLAGCTESSHALNISTPQEAPQEVQPPVAKSLPSSLLLSWNPPKKANGIITQYCLYMDGRLIYSGSEENYTVTDLAVFTPHQFLLSACTHVGCTNSSWVLLYTAQLPPEHVDSPVLTVLDSRTIHIQWKQPRKISGILERYVLYMSNHTHDFTIWSVIYNSTELFQDHMLQYVLPGNKYLIKLGACTGGGCTVSEASEALTDEDIPEGVPAPKAHSYSPDSFNVSWTEPEYPNGVITSYGLYLDGILIHNSSELSYRAYGFAPWSLHSFRVQACTAKGCALGPLVENRTLEAPPEGTVNVFVKTQGSRKAHVRWEAPFRPNGLLTHSVLFTGIFYVDPVGNNYTLLNVTKVMYSGEETNLWVLIDGLVPFTNYTVQVNISNSQGSLITDPITIAMPPGAPDGVLPPRLSSATPTSLQVVWSTPARNNAPGSPRYQLQMRSGDSTHGFLELFSNPSASLSYEVSDLQPYTEYMFRLVASNGFGSAHSSWIPFMTAEDKPGPVVPPILLDVKSRMMLVTWQHPRKSNGVITHYNIYLHGRLYLRTPGNVTNCTVMHLHPYTAYKFQVEACTSKGCSLSPESQTVWTLPGAPEGIPSPELFSDTPTSVIISWQPPTHPNGLVENFTIERRVKGKEEVTTLVTLPRSHSMRFIDKTSALSPWTKYEYRVLMSTLHGGTNSSAWVEVTTRPSRPAGVQPPVVTVLEPDAVQVTWKPPLIQNGDILSYEIHMPDPHITLTNVTSAVLSQKVTHLIPFTNYSVTIVACSGGNGYLGGCTESLPTYVTTHPTVPQNVGPLSVIPLSESYVVISWQPPSKPNGPNLRYELLRRKIQQPLASNPPEDLNRWHNIYSGTQWLYEDKGLSRFTTYEYMLFVHNSVGFTPSREVTVTTLAGLPERGANLTASVLNHTAIDVRWAKPTVQDLQGEVEYYTLFWSSATSNDSLKILPDVNSHVIGHLKPNTEYWIFISVFNGVHSINSAGLHATTCDGEPQGMLPPEVVIINSTAVRVIWTSPSNPNGVVTEYSIYVNNKLYKTGMNVPGSFILRDLSPFTIYDIQVEVCTIYACVKSNGTQITTVEDTPSDIPTPTIRGITSRSLQIDWVSPRKPNGIILGYDLLWKTWYPCAKTQKLVQDQSDELCKAVRCQKPESICGHICYSSEAKVCCNGVLYNPKPGHRCCEEKYIPFVLNSTGVCCGGRIQEAQPNHQCCSGYYARILPGEVCCPDEQHNRVSVGIGDSCCGRMPYSTSGNQICCAGRLHDGHGQKCCGRQIVSNDLECCGGEEGVVYNRLPGMFCCGQDYVNMSDTICCSASSGESKAHIKKNDPVPVKCCETELIPKSQKCCNGVGYNPLKYVCSDKISTGMMMKETKECRILCPASMEATEHCGRCDFNFTSHICTVIRGSHNSTGKASIEEMCSSAEETIHTGSVNTYSYTDVNLKPYMTYEYRISAWNSYGRGLSKAVRARTKEDVPQGVSPPTWTKIDNLEDTIVLNWRKPIQSNGPIIYYILLRNGIERFRGTSLSFSDKEGIQPFQEYSYQLKACTVAGCATSSKVVAATTQGVPESILPPSITALSAVALHLSWSVPEKSNGVIKEYQIRQVGKGLIHTDTTDRRQHTVTGLQPYTNYSFTLTACTSAGCTSSEPFLGQTLQAAPEGVWVTPRHIIINSTTVELYWSLPEKPNGLVSQYQLSRNGNLLFLGGSEEQNFTDKNLEPNSRYTYKLEVKTGGGSSASDDYIVQTPMSTPEEIYPPYNITVIGPYSIFVAWIPPGILIPEIPVEYNVLLNDGSVTPLAFSVGHHQSTLLENLTPFTQYEIRIQACQNGSCGVSSRMFVKTPEAAPMDLNSPVLKALGSACIEIKWMPPEKPNGIIINYFIYRRPAGIEEESVLFVWSEGALEFMDEGDTLRPFTLYEYRVRACNSKGSVESLWSLTQTLEAPPQDFPAPWAQATSAHSVLLNWTKPESPNGIISHYRVVYQERPDDPTFNSPTVHAFTVKGTSHQAHLYGLEPFTTYRIGVVAANHAGEILSPWTLIQTLESSPSGLRNFIVEQKENGRALLLQWSEPMRTNGVIKTYNIFSDGFLEYSGLNRQFLFRRLDPFTLYTLTLEACTRAGCAHSAPQPLWTDEAPPDSQLAPTVHSVKSTSVELSWSEPVNPNGKIIRYEVIRRCFEGKAWGNQTIQADEKIVFTEYNTERNTFMYNDTGLQPWTQCEYKIYTWNSAGHTCSSWNVVRTLQAPPEGLSPPVISYVSMNPQKLLISWIPPEQSNGIIQSYRLQRNEMLYPFSFDPVTFNYTDEELLPFSTYSYALQACTSGGCSTSKPTSITTLEAAPSEVSPPDLWAVSATQMNVCWSPPTVQNGKITKYLVRYDNKESLAGQGLCLLVSHLQPYSQYNFSLVACTNGGCTASVSKSAWTMEALPENMDSPTLQVTGSESIEITWKPPRNPNGQIRSYELRRDGTIVYTGLETRYRDFTLTPGVEYSYTVTASNSQGGILSPLVKDRTSPSAPSGMEPPKLQARGPQEILVNWDPPVRTNGDIINYTLFIRELFERETKIIHINTTHNSFGMQSYIVNQLKPFHRYEIRIQACTTLGCASSDWTFIQTPEIAPLMQPPPHLEVQMAPGGFQPTVSLLWTGPLQPNGKVLYYELYRRQIATQPRKSNPVLIYNGSSTSFIDSELLPFTEYEYQVWAVNSAGKAPSSWTWCRTGPAPPEGLRAPTFHVISSTQAVVNISAPGKPNGIVSLYRLFSSSAHGAETVLSEGMATQQTLHGLQAFTNYSIGVEACTCFNCCSKGPTAELRTHPAPPSGLSSPQIGTLASRTASFRWSPPMFPNGVIHSYELQFHVACPPDSALPCTPSQIETKYTGLGQKASLGGLQPYTTYKLRVVAHNEVGSTASEWISFTTQKELPQYRAPFSVDSNLSVVCVNWSDTFLLNGQLKEYVLTDGGRRVYSGLDTTLYIPRTADKTFFFQVICTTDEGSVKTPLIQYDTSTGLGLVLTTPGKKKGSRSKSTEFYSELWFIVLMAMLGLILLAIFLSLILQRKIHKEPYIRERPPLVPLQKRMSPLNVYPPGENHMGLADTKIPRSGTPVSIRSNRSACVLRIPSQNQTSLTYSQGSLHRSVSQLMDIQDKKVLMDNSLWEAIMGHNSGLYVDEEDLMNAIKDFSSVTKERTTFTDTHL

SEQ ID NO: 3 - DNA, 22 bp, synthetic construct
  misc_feature 1..22: note = Description of Artificial Sequence: Synthetic oligonucleotide
  source 1..22: mol_type = other DNA
ggaatgcagtactgctgaacgg

SEQ ID NO: 4 - DNA, 62 bp, synthetic construct
  misc_feature 1..62: note = Description of Artificial Sequence: Synthetic oligonucleotide
  source 1..62: mol_type = other DNA
tgcaccattgggaatgcggaggggtggacacgggggtggctacctggacatcggcaatgtgg

SEQ ID NO: 5 - DNA, 63 bp, synthetic construct
  misc_feature 1..63: note = Description of Artificial Sequence: Synthetic oligonucleotide
  source 1..63: mol_type = other DNA
tgcaccattgggaatgcagtactgctggacacgggggtggctacctggacatcggcaatgtgg

SEQ ID NO: 6 - DNA, 75 bp, synthetic construct
  misc_feature 1..75: note = Description of Artificial Sequence: Synthetic oligonucleotide
  source 1..75: mol_type = other DNA
tgcaccattgggaatgcagtactgctgaacggaggggtggacacgggggtggctacctggacatcggcaatgtgg

SEQ ID NO: 7 - DNA, 38 bp, synthetic construct
  misc_feature 1..38: note = Description of Artificial Sequence: Synthetic oligonucleotide
  source 1..38: mol_type = other DNA
ttgggaatgcagtactgctggacacgggggtggctacc

SEQ ID NO: 8 - DNA, 43 bp, synthetic construct
  misc_feature 1..43: note = Description of Artificial Sequence: Synthetic oligonucleotide
  source 1..43: mol_type = other DNA
ttgggaatgcagtactgcaggggtggacacgggggtggctacc

SEQ ID NO: 9 - DNA, 37 bp, synthetic construct
  misc_feature 1..37: note = Description of Artificial Sequence: Synthetic oligonucleotide
  source 1..37: mol_type = other DNA
ttgggaatgcggaggggtggacacgggggtggctacc

SEQ ID NO: 10 - DNA, 43 bp, synthetic construct
  misc_feature 1..43: note = Description of Artificial Sequence: Synthetic oligonucleotide
  source 1..43: mol_type = other DNA
ttgggaatgcagtactggaggggtggacacgggggtggctacc

SEQ ID NO: 11 - DNA, 49 bp, synthetic construct
  misc_feature 1..49: note = Description of Artificial Sequence: Synthetic oligonucleotide
  source 1..49: mol_type = other DNA
ttgggaatgcagtactgctgaaggaggggtggacacgggggtggctacc

SEQ ID NO: 12 - DNA, 23 bp, synthetic construct
  misc_feature 1..23: note = Description of Artificial Sequence: Synthetic oligonucleotide
  source 1..23: mol_type = other DNA
acctccgagaggacccctccagg

SEQ ID NO: 13 - DNA, 23 bp, synthetic construct
  misc_feature 1..23: note = Description of Artificial Sequence: Synthetic oligonucleotide
  source 1..23: mol_type = other DNA
atttagctctactaagcgagagg

SEQ ID NO: 14 - DNA, 23 bp, synthetic construct
  misc_feature 1..23: note = Description of Artificial Sequence: Synthetic oligonucleotide
  source 1..23: mol_type = other DNA
ggatgattcgtgactgcttgagg

SEQ ID NO: 15 - DNA, 25 bp, synthetic construct
  misc_feature 1..25: note = Description of Artificial Sequence: Synthetic oligonucleotide
  source 1..25: mol_type = other DNA
acgtcaaatagctcggtttggatgg

SEQ ID NO: 16 - DNA, 23 bp, synthetic construct
  misc_feature 1..23: note = Description of Artificial Sequence: Synthetic oligonucleotide
  source 1..23: mol_type = other DNA
ggggaaaggagccactttagagg

SEQ ID NO: 17 - DNA, 23 bp, synthetic construct
  misc_feature 1..23: note = Description of Artificial Sequence: Synthetic oligonucleotide
  source 1..23: mol_type = other DNA
ggtatcataaggatccatctagg

SEQ ID NO: 18 - DNA, 58 bp, synthetic construct
  misc_feature 1..58: note = Description of Artificial Sequence: Synthetic oligonucleotide
  source 1..58: mol_type = other DNA
tcctcaccttttaaatatattttatctttagggcttaggtgtgatcattgcaattttg

SEQ ID NO: 19 - DNA, 58 bp, synthetic construct
  misc_feature 1..58: note = Description of Artificial Sequence: Synthetic oligonucleotide
  source 1..58: mol_type = other DNA
tcctcaccttttaaatatattttatctttagggcttaggtgtgatcgttgcaattttg

SEQ ID NO: 20 - DNA, 58 bp, synthetic construct; identical to SEQ ID NO: 19
  misc_feature 1..58: note = Description of Artificial Sequence: Synthetic oligonucleotide
  source 1..58: mol_type = other DNA

SEQ ID NO: 21 - RNA, 102 nt, synthetic construct
  misc_feature 1..102: note = Description of Artificial Sequence: Synthetic polynucleotide
  modified_base 1..20: mod_base = OTHER; note = a, c, u, g, unknown or other
  source 1..102: mol_type = other RNA
nnnnnnnnnnnnnnnnnnnngttttagtactctggaaacagaatctactaaaacaaggcaaaatgccgtgtttatctcgtcaacttgttggcgagatttttt

SEQ ID NO: 22 - protein, 7 aa, synthetic construct
  REGION 1..7: note = Description of Artificial Sequence: Synthetic peptide
PKKKRKV

SEQ ID NO: 23 - protein, 7 aa, synthetic construct
  REGION 1..7: note = Description of Artificial Sequence: Synthetic peptide
PKKKRRV

SEQ ID NO: 24 - protein, 16 aa, synthetic construct
  REGION 1..16: note = Description of Artificial Sequence: Synthetic peptide
KRPAATKKAGQAKKKK

SEQ ID NO: 25 - DNA, 60 bp, synthetic construct
  misc_feature 1..60: note = Description of Artificial Sequence: Synthetic oligonucleotide
  source 1..60: mol_type = other DNA
tagcaataaaggatcgtttattttcattggaagcgtgtgttggttttttgatcaggcgcg

SEQ ID NO: 26 - DNA, 106 bp, synthetic construct
  misc_feature 1..106: note = Description of Artificial Sequence: Synthetic polynucleotide
  modified_base 1..24: mod_base = OTHER; note = a, c, t, g, unknown or other
  misc_feature 1..24: note = /note="This region may encompass 16-24 nucleotides"
  source 1..106: mol_type = other DNA
nnnnnnnnnnnnnnnnnnnnnnnngttttagtactctggaaacagaatctactaaaacaaggcaaaatgccgtgtttatctcgtcaacttgttggcgagatttttt

SEQ ID NO: 27 - RNA, 106 nt, synthetic construct
  misc_feature 1..106: note = Description of Artificial Sequence: Synthetic polynucleotide
  modified_base 1..24: mod_base = OTHER; note = a, c, u, g, unknown or other
  misc_feature 1..24: note = /note="This region may encompass 16-24 nucleotides"
  source 1..106: mol_type = other RNA
nnnnnnnnnnnnnnnnnnnnnnnngttttagtactctggaaacagaatctactaaaacaaggcaaaatgccgtgtttatctcgtcaacttgttggcgagatttttt

SEQ ID NO: 28 - DNA, 106 bp, synthetic construct
  misc_feature 1..106: note = Description of Artificial Sequence: Synthetic polynucleotide
  modified_base 1..24: mod_base = OTHER; note = a, c, t, g, unknown or other
  misc_feature 1..24: note = /note="This region may encompass 16-24 nucleotides"
  source 1..106: mol_type = other DNA
nnnnnnnnnnnnnnnnnnnnnnnngttatagtactctggaaacagaatctactataacaaggcaaaatgccgtgtttatctcgtcaacttgttggcgagatttttt

SEQ ID NO: 29 - RNA, 106 nt, synthetic construct
  misc_feature 1..106: note = Description of Artificial Sequence: Synthetic polynucleotide
  modified_base 1..24: mod_base = OTHER; note = a, c, u, g, unknown or other
  misc_feature 1..24: note = /note="This region may encompass 16-24 nucleotides"
  source 1..106: mol_type = other RNA
nnnnnnnnnnnnnnnnnnnnnnnngttatagtactctggaaacagaatctactataacaaggcaaaatgccgtgtttatctcgtcaacttgttggcgagatttttt

SEQ ID NO: 30 - DNA, 20 bp, synthetic construct
  misc_feature 1..20: note = Description of Artificial Sequence: Synthetic oligonucleotide
  source 1..20: mol_type = other DNA
gagagcatgatttatattaa

SEQ ID NO: 31 - DNA, 20 bp, synthetic construct
  misc_feature 1..20: note = Description of Artificial Sequence: Synthetic oligonucleotide
  source 1..20: mol_type = other DNA
ggccccctatggcattgctt

SEQ ID NO: 32 - DNA, 20 bp, synthetic construct
  misc_feature 1..20: note = Description of Artificial Sequence: Synthetic oligonucleotide
  source 1..20: mol_type = other DNA
gtccttttttattttcctta

SEQ ID NO: 33 - DNA, 20 bp, synthetic construct
  misc_feature 1..20: note = Description of Artificial Sequence: Synthetic oligonucleotide
  source 1..20: mol_type = other DNA
gtgatggatacattaattag

SEQ ID NO: 34 - DNA, 20 bp, synthetic construct
  misc_feature 1..20: note = Description of Artificial Sequence: Synthetic oligonucleotide
  source 1..20: mol_type = other DNA
ggatatttggaaactatcta

SEQ ID NO: 35 - DNA, 20 bp, synthetic construct
  misc_feature 1..20: note = Description of Artificial Sequence: Synthetic oligonucleotide
  source 1..20: mol_type = other DNA
gcatatcatttaatttcaat

SEQ ID NO: 36 - DNA, 20 bp, synthetic construct
  misc_feature 1..20: note = Description of Artificial Sequence: Synthetic oligonucleotide
  source 1..20: mol_type = other DNA
gtagaaaagcatttcctaaa

SEQ ID NO: 37 - DNA, 20 bp, synthetic construct
  misc_feature 1..20: note = Description of Artificial Sequence: Synthetic oligonucleotide
  source 1..20: mol_type = other DNA
gtcagctgataactattttt

SEQ ID NO: 38 - DNA, 20 bp, synthetic construct
  misc_feature 1..20: note = Description of Artificial Sequence: Synthetic oligonucleotide
  source 1..20: mol_type = other DNA
gtacttatcatgtttttggg

SEQ ID NO: 39 - DNA, 21 bp, synthetic construct
  misc_feature 1..21: note = Description of Artificial Sequence: Synthetic oligonucleotide
  source 1..21: mol_type = other DNA
gaaaagcatttcctaaactgg

SEQ ID NO: 40 - DNA, 21 bp, synthetic construct
  misc_feature 1..21: note = Description of Artificial Sequence: Synthetic oligonucleotide
  source 1..21: mol_type = other DNA
gcatatcatttaatttcaata

SEQ ID NO: 41 - DNA, 21 bp, synthetic construct
  misc_feature 1..21: note = Description of Artificial Sequence: Synthetic oligonucleotide
  source 1..21: mol_type = other DNA
ggagagcatgatttatattaa

SEQ ID NO: 42 - DNA, 21 bp, synthetic construct
  misc_feature 1..21: note = Description of Artificial Sequence: Synthetic oligonucleotide
  source 1..21: mol_type = other DNA
gaacttattcattctgtctag

SEQ ID NO: 43 - DNA, 21 bp, synthetic construct
  misc_feature 1..21: note = Description of Artificial Sequence: Synthetic oligonucleotide
  source 1..21: mol_type = other DNA
gttatttaaattcatggatat

SEQ ID NO: 44 - DNA, 21 bp, synthetic construct
  misc_feature 1..21: note = Description of Artificial Sequence: Synthetic oligonucleotide
  source 1..21: mol_type = other DNA
ggcatatcatttaatttcaat

SEQ ID NO: 45 - DNA, 21 bp, synthetic construct
  misc_feature 1..21: note = Description of Artificial Sequence: Synthetic oligonucleotide
  source 1..21: mol_type = other DNA
gccccctatggcattgcttgt

SEQ ID NO: 46 - DNA, 21 bp, synthetic construct
  misc_feature 1..21: note = Description of Artificial Sequence: Synthetic oligonucleotide
  source 1..21: mol_type = other DNA
ggtccttttttattttcctta

SEQ ID NO: 47 - DNA, 21 bp, synthetic construct
  misc_feature 1..21: note = Description of Artificial Sequence: Synthetic oligonucleotide
  source 1..21: mol_type = other DNA
ggtgatggatacattaattag

SEQ ID NO: 48 - DNA, 22 bp, synthetic construct
  misc_feature 1..22: note = Description of Artificial Sequence: Synthetic oligonucleotide
  source 1..22: mol_type = other DNA
gttatttaaattcatggatatt

SEQ ID NO: 49 - DNA, 22 bp, synthetic construct
  misc_feature 1..22: note = Description of Artificial Sequence: Synthetic oligonucleotide
  source 1..22: mol_type = other DNA
gtttgtgtctcgtctatcttga

SEQ ID NO: 50 - DNA, 22 bp, synthetic construct
  misc_feature 1..22: note = Description of Artificial Sequence: Synthetic oligonucleotide
  source 1..22: mol_type = other DNA
gataaaagggtattacaaggca

SEQ ID NO: 51 - DNA, 22 bp, synthetic construct
  misc_feature 1..22: note = Description of Artificial Sequence: Synthetic oligonucleotide
  source 1..22: mol_type = other DNA
ggccccctatggcattgcttgt

SEQ ID NO: 52 - DNA, 22 bp, synthetic construct
  misc_feature 1..22: note = Description of Artificial Sequence: Synthetic oligonucleotide
  source 1..22: mol_type = other DNA
ggcatatcatttaatttcaata

SEQ ID NO: 53 - DNA, 22 bp, synthetic construct
  misc_feature 1..22: note = Description of Artificial Sequence: Synthetic oligonucleotide
  source 1..22: mol_type = other DNA
gaaaagcatttcctaaactgga

SEQ ID NO: 54 - DNA, 20 bp, synthetic construct
  misc_feature 1..20: note = Description of Artificial Sequence: Synthetic oligonucleotide
  source 1..20: mol_type = other DNA
gaatttaaataactcactgc

SEQ ID NO: 55 - DNA, 20 bp, synthetic construct
  misc_feature 1..20: note = Description of Artificial Sequence: Synthetic oligonucleotide
  source 1..20: mol_type = other DNA
gcttttctacatatgagttc

SEQ ID NO: 56 - DNA, 20 bp, synthetic construct
  misc_feature 1..20: note = Description of Artificial Sequence: Synthetic oligonucleotide
  source 1..20: mol_type = other DNA
gatgatacgaacacaaaata

SEQ ID NO: 57 - DNA, 20 bp, synthetic construct
  misc_feature 1..20: note = Description of Artificial Sequence: Synthetic oligonucleotide
  source 1..20: mol_type = other DNA
ggattaaaccaaaaattgcc

SEQ ID NO: 58 - DNA, 20 bp, synthetic construct
  misc_feature 1..20: note = Description of Artificial Sequence: Synthetic oligonucleotide
  source 1..20: mol_type = other DNA
ggagtacacatatacatttt

SEQ ID NO: 59 - DNA, 20 bp, synthetic construct
  misc_feature 1..20: note = Description of Artificial Sequence: Synthetic oligonucleotide
  source 1..20: mol_type = other DNA
gttaaagaacttgccttcat

SEQ ID NO: 60 - DNA, 20 bp, synthetic construct
  misc_feature 1..20: note = Description of Artificial Sequence: Synthetic oligonucleotide
  source 1..20: mol_type = other DNA
gtgctcatttaaaattatag

SEQ ID NO: 61 - DNA, 20 bp, synthetic construct
  misc_feature 1..20: note = Description of Artificial Sequence: Synthetic oligonucleotide
  source 1..20: mol_type = other DNA
gcagtgagttatttaaattc

SEQ ID NO: 62 - DNA, 21 bp, synthetic construct
  misc_feature 1..21: note = Description of Artificial Sequence: Synthetic oligonucleotide
  source 1..21: mol_type = other DNA
gatgtttaataaaaggttaag

SEQ ID NO: 63 - DNA, 21 bp, synthetic construct
  misc_feature 1..21: note = Description of Artificial Sequence: Synthetic oligonucleotide
  source 1..21: mol_type = other DNA
gtgatggatacattaattagc

SEQ ID NO: 64 - DNA, 21 bp, synthetic construct
  misc_feature 1..21: note = Description of Artificial Sequence: Synthetic oligonucleotide
  source 1..21: mol_type = other DNA
gataaaatatatttaaaaggt

SEQ ID NO: 65 - DNA, 22 bp, synthetic construct
  misc_feature 1..22: note = Description of Artificial Sequence: Synthetic oligonucleotide
  source 1..22: mol_type = other DNA
gtaaggttattctaaaagataa

SEQ ID NO: 66 - DNA, 22 bp, synthetic construct
  misc_feature 1..22: note = Description of Artificial Sequence: Synthetic oligonucleotide
  source 1..22: mol_type = other DNA
gaacttgccttcattggagttc

SEQ ID NO: 67 - DNA, 22 bp, synthetic construct
  misc_feature 1..22: note = Description of Artificial Sequence: Synthetic oligonucleotide
  source 1..22: mol_type = other DNA
ggtgatggatacattaattagc

SEQ ID NO: 68 - DNA, 22 bp, synthetic construct
  misc_feature 1..22: note = Description of Artificial Sequence: Synthetic oligonucleotide
  source 1..22: mol_type = other DNA
gaaattaaatgatatgccttag

SEQ ID NO: 69 - DNA, 22 bp, synthetic construct
  misc_feature 1..22: note = Description of Artificial Sequence: Synthetic oligonucleotide
  source 1..22: mol_type = other DNA
gaaggcaagttctttaacagtg

SEQ ID NO: 70 - DNA, 22 bp, synthetic construct
  misc_feature 1..22: note = Description of Artificial Sequence: Synthetic oligonucleotide
  source 1..22: mol_type = other DNA
gataaaatagaggagcatacaa

SEQ ID NO: 71 - DNA, 20 bp, synthetic construct
  misc_feature 1..20: note = Description of Artificial Sequence: Synthetic oligonucleotide
  source 1..20: mol_type = other DNA
gtccccttctgagagagaga

SEQ ID NO: 72 - DNA, 20 bp, synthetic construct
  misc_feature 1..20: note = Description of Artificial Sequence: Synthetic oligonucleotide
  source 1..20: mol_type = other DNA
ggtctatccctctcccaatt

SEQ ID NO: 73 - DNA, 20 bp, synthetic construct
  misc_feature 1..20: note = Description of Artificial Sequence: Synthetic oligonucleotide
  source 1..20: mol_type = other DNA
ggggtctatccctctcccaa

SEQ ID NO: 74 - DNA, 20 bp, synthetic construct
  misc_feature 1..20: note = Description of Artificial Sequence: Synthetic oligonucleotide
  source 1..20: mol_type = other DNA
gaaagataagtttgtatata

SEQ ID NO: 75 - DNA, 20 bp, synthetic construct
  misc_feature 1..20: note = Description of Artificial Sequence: Synthetic oligonucleotide
  source 1..20: mol_type = other DNA
gccatatacccatgtagaga

SEQ ID NO: 76 - DNA, 20 bp, synthetic construct
  misc_feature 1..20: note = Description of Artificial Sequence: Synthetic oligonucleotide
  source 1..20: mol_type = other DNA
gaggtaaagtccccttctga

SEQ ID NO: 77 - DNA, 20 bp, synthetic construct
  misc_feature 1..20: note = Description of Artificial Sequence: Synthetic oligonucleotide
  source 1..20: mol_type = other DNA
ggtggccatatacccatgta

SEQ ID NO: 78 - DNA, 20 bp, synthetic construct
  misc_feature 1..20: note = Description of Artificial Sequence: Synthetic oligonucleotide
  source 1..20: mol_type = other DNA
ggaccactgcagtcaggact

SEQ ID NO: 79 - DNA, 20 bp, synthetic construct
  misc_feature 1..20: note = Description of Artificial Sequence: Synthetic oligonucleotide
  source 1..20: mol_type = other DNA
gaagccacaaaccagaaaca

SEQ ID NO: 80 - DNA, 20 bp, synthetic construct
  misc_feature 1..20: note = Description of Artificial Sequence: Synthetic oligonucleotide
  source 1..20: mol_type = other DNA
gaagttacctaagttaacaa

SEQ ID NO: 81 - DNA, 20 bp, synthetic construct
  misc_feature 1..20: note = Description of Artificial Sequence: Synthetic oligonucleotide
  source 1..20: mol_type = other DNA
gtagaaattgagtctcaatt

SEQ ID NO: 82 - DNA, 20 bp, synthetic construct
  misc_feature 1..20: note = Description of Artificial Sequence: Synthetic oligonucleotide
  source 1..20: mol_type = other DNA
gtaatcagtgtcaaccaggt

SEQ ID NO: 83 - DNA, 20 bp, synthetic construct
  misc_feature 1..20: note = Description of Artificial Sequence: Synthetic oligonucleotide
  source 1..20: mol_type = other DNA
gtggtaagtatcccagaaga

SEQ ID NO: 84 - DNA, 20 bp, synthetic construct
  misc_feature 1..20: note = Description of Artificial Sequence: Synthetic oligonucleotide
  source 1..20: mol_type = other DNA
gagaggtaaagtccccttct

SEQ ID NO: 85 - DNA, 20 bp, synthetic construct
  misc_feature 1..20: note = Description of Artificial Sequence: Synthetic oligonucleotide
  source 1..20: mol_type = other DNA
gtagaattataaacaatttc

SEQ ID NO: 86 - DNA, 20 bp, synthetic construct
  misc_feature 1..20: note = Description of Artificial Sequence: Synthetic oligonucleotide
  source 1..20: mol_type = other DNA
ggtaaagtccccttctgaga

SEQ ID NO: 87 - DNA, 20 bp, synthetic construct
  misc_feature 1..20: note = Description of Artificial Sequence: Synthetic oligonucleotide
  source 1..20: mol_type = other DNA
gggtctatccctctcccaat

SEQ ID NO: 88 - DNA, 20 bp, synthetic construct
  misc_feature 1..20: note = Description of Artificial Sequence: Synthetic oligonucleotide
  source 1..20: mol_type = other DNA
gagagaggtaaagtcccctt

SEQ ID NO: 89 - DNA, 21 bp, synthetic construct
  misc_feature 1..21: note = Description of Artificial Sequence: Synthetic oligonucleotide
  source 1..21: mol_type = other DNA
gtaaagtccccttctgagaga

SEQ ID NO: 90 - DNA, 21 bp, synthetic construct
  misc_feature 1..21: note = Description of Artificial Sequence: Synthetic oligonucleotide
  source 1..21: mol_type = other DNA
gggtctatccctctcccaatt

SEQ ID NO: 91 - DNA, 21 bp, synthetic construct
  misc_feature 1..21: note = Description of Artificial Sequence: Synthetic oligonucleotide
  source 1..21: mol_type = other DNA
gggtggccatatacccatgta

SEQ ID NO: 92 - DNA, 21 bp, synthetic construct
  misc_feature 1..21: note = Description of Artificial Sequence: Synthetic oligonucleotide
  source 1..21: mol_type = other DNA
gctatatgttctagttttata

SEQ ID NO: 93 - DNA, 21 bp, synthetic construct
  misc_feature 1..21: note = Description of Artificial Sequence: Synthetic oligonucleotide
  source 1..21: mol_type = other DNA
gatataaatacagtaatgatt

SEQ ID NO: 94 - DNA, 21 bp, synthetic construct
  misc_feature 1..21: note = Description of Artificial Sequence: Synthetic oligonucleotide
  source 1..21: mol_type = other DNA
gagacaaatgaatatgtatca

SEQ ID NO: 95 - DNA, 21 bp, synthetic construct
  misc_feature 1..21: note = Description of Artificial Sequence: Synthetic oligonucleotide
  source 1..21: mol_type = other DNA
ggccatatacccatgtagaga

SEQ ID NO: 96 - DNA, 21 bp, synthetic construct
  misc_feature 1..21: note = Description of Artificial Sequence: Synthetic oligonucleotide
  source 1..21: mol_type = other DNA
gagtcaattcgaattttcctc

SEQ ID NO: 97 - DNA, 21 bp, synthetic construct
  misc_feature 1..21: note = Description of Artificial Sequence: Synthetic oligonucleotide
  source 1..21: mol_type = other DNA
ggtggtaagtatcccagaaga

SEQ ID NO: 98 - DNA, 21 bp, synthetic construct
  misc_feature 1..21: note = Description of Artificial Sequence: Synthetic oligonucleotide
  source 1..21: mol_type = other DNA
gtagaagccacaaaccagaaa

SEQ ID NO: 99 - DNA, 21 bp, synthetic construct
  misc_feature 1..21: note = Description of Artificial Sequence: Synthetic oligonucleotide
  source 1..21: mol_type = other DNA
ggtagaattataaacaatttc

SEQ ID NO: 100 - DNA, 21 bp, synthetic construct
  misc_feature 1..21: note = Description of Artificial Sequence: Synthetic oligonucleotide
  source 1..21: mol_type = other DNA
gtcaattttattttccagaga

SEQ ID NO: 101 - DNA, 21 bp, synthetic construct
  misc_feature 1..21: note = Description of Artificial Sequence: Synthetic oligonucleotide
  source 1..21: mol_type = other DNA
ggaaagataagtttgtatata

SEQ ID NO: 102 - DNA, 21 bp, synthetic construct
  misc_feature 1..21: note = Description of Artificial Sequence: Synthetic oligonucleotide
  source 1..21: mol_type = other DNA
ggggtctatccctctcccaat

SEQ ID NO: 103 - DNA, 21 bp, synthetic construct
  misc_feature 1..21: note = Description of Artificial Sequence: Synthetic oligonucleotide
  source 1..21: mol_type = other DNA
gtgtaagatcaaagagacaag

SEQ ID NO: 104 - DNA, 22 bp, synthetic construct
  misc_feature 1..22: note = Description of Artificial Sequence: Synthetic oligonucleotide
  source 1..22: mol_type = other DNA
gtccccttctgagagagagaga

SEQ ID NO: 105 - DNA, 22 bp, synthetic construct
  misc_feature 1..22: note = Description of Artificial Sequence: Synthetic oligonucleotide
  source 1..22: mol_type = other DNA
gatataaatacagtaatgattt

SEQ ID NO: 106 - DNA, 22 bp, synthetic construct
  misc_feature 1..22: note = Description of Artificial Sequence: Synthetic oligonucleotide
  source 1..22: mol_type = other DNA
ggggtctatccctctcccaatt

SEQ ID NO: 107 - DNA, 22 bp, synthetic construct
  misc_feature 1..22: note = Description of Artificial Sequence: Synthetic oligonucleotide
  source 1..22: mol_type = other DNA
ggctatatgttctagttttata

SEQ ID NO: 108 - DNA, 22 bp, synthetic construct
  misc_feature 1..22: note = Description of Artificial Sequence: Synthetic oligonucleotide
  source 1..22: mol_type = other DNA
gtgtagaaattgagtctcaatt

SEQ ID NO: 109 - DNA, 22 bp, synthetic construct
  misc_feature 1..22: note = Description of Artificial Sequence: Synthetic oligonucleotide
  source 1..22: mol_type = other DNA
gagagaggtaaagtccccttct

SEQ ID NO: 110 - DNA, 22 bp, synthetic construct
  misc_feature 1..22: note = Description of Artificial Sequence: Synthetic oligonucleotide
  source 1..22: mol_type = other DNA
ggtaaagtccccttctgagaga

SEQ ID NO: 111 - DNA, 22 bp, synthetic construct
  misc_feature 1..22: note = Description of Artificial Sequence: Synthetic oligonucleotide
  source 1..22: mol_type = other DNA
gccgatcggatttatttcataa

SEQ ID NO: 112 - DNA, 22 bp, synthetic construct
  misc_feature 1..22: note = Description of Artificial Sequence: Synthetic oligonucleotide
  source 1..22: mol_type = other DNA
gatttttaaaaaactgttaaaa

SEQ ID NO: 113 - DNA, 22 bp, synthetic construct
  misc_feature 1..22: note = Description of Artificial Sequence: Synthetic oligonucleotide
  source 1..22: mol_type = other DNA
gccatatacccatgtagagaaa

SEQ ID NO: 114 - DNA, 22 bp, synthetic construct
  misc_feature 1..22: note = Description of Artificial Sequence: Synthetic oligonucleotide
  source 1..22: mol_type = other DNA
gagaagttacctaagttaacaa

SEQ ID NO: 115 - DNA, 22 bp, synthetic construct
  misc_feature 1..22: note = Description of Artificial Sequence: Synthetic oligonucleotide
  source 1..22: mol_type = other DNA
gtgtaatcagtgtcaaccaggt

SEQ ID NO: 116 - DNA, 22 bp, synthetic construct
  misc_feature 1..22: note = Description of Artificial Sequence: Synthetic oligonucleotide
  source 1..22: mol_type = other DNA
gtcaattttattttccagagaa

SEQ ID NO: 117 - DNA, 22 bp, synthetic construct
  misc_feature 1..22: note = Description of Artificial Sequence: Synthetic oligonucleotide
  source 1..22: mol_type = other DNA
gagaggtaaagtccccttctga

SEQ ID NO: 118 - DNA, 22 bp, synthetic construct
  misc_feature 1..22: note = Description of Artificial Sequence: Synthetic oligonucleotide
  source 1..22: mol_type = other DNA
gaggtaaagtccccttctgaga

SEQ ID NO: 119 - DNA, 22 bp, synthetic construct
  misc_feature 1..22: note = Description of Artificial Sequence: Synthetic oligonucleotide
  source 1..22: mol_type = other DNA
gtatatggccaccctatgtccc

SEQ ID NO: 120 - DNA, 22 bp, synthetic construct
  misc_feature 1..22: note = Description of Artificial Sequence: Synthetic oligonucleotide
  source 1..22: mol_type = other DNA
gtctccataatcttcctgtctt

SEQ ID NO: 121 - DNA, 20 bp, synthetic construct
  misc_feature 1..20: note = Description of Artificial Sequence: Synthetic oligonucleotide
  source 1..20: mol_type = other DNA
gttaaatagttatatatgtg

SEQ ID NO: 122 - DNA, 20 bp, synthetic construct
  misc_feature 1..20: note = Description of Artificial Sequence: Synthetic oligonucleotide
  source 1..20: mol_type = other DNA
gaccactgcagtcaggactc

SEQ ID NO: 123 - DNA, 20 bp, synthetic construct
  misc_feature 1..20: note = Description of Artificial Sequence: Synthetic oligonucleotide
  source 1..20: mol_type = other DNA
gtaagatcaaagagacaaga

SEQ ID NO: 124 - DNA, 20 bp, synthetic construct
  misc_feature 1..20: note = Description of Artificial Sequence: Synthetic oligonucleotide
  source 1..20: mol_type = other DNA
gggtgtcacgtacttataaa

SEQ ID NO: 125 - DNA, 20 bp, synthetic construct
  misc_feature 1..20: note = Description of Artificial Sequence: Synthetic oligonucleotide
  source 1..20: mol_type = other DNA
gagacaagaaggaattgatg

SEQ ID NO: 126 - DNA, 21 bp, synthetic construct
  misc_feature 1..21: note = Description of Artificial Sequence: Synthetic oligonucleotide
  source 1..21: mol_type = other DNA
gatttacttcaagtgtagaaa

SEQ ID NO: 127 - DNA, 21 bp, synthetic construct
  misc_feature 1..21: note = Description of Artificial Sequence: Synthetic oligonucleotide
  source 1..21: mol_type = other DNA
gtccttctccttaggttttta

SEQ ID NO: 128 - DNA, 21 bp, synthetic construct
  misc_feature 1..21: note = Description of Artificial Sequence: Synthetic oligonucleotide
  source 1..21: mol_type = other DNA
gcatggcccaattatcctagg

SEQ ID NO: 129 - DNA, 21 bp, synthetic construct
  misc_feature 1..21: note = Description of Artificial Sequence: Synthetic oligonucleotide
  source 1..21: mol_type = other DNA
gtgtgatttgcttgccagaga

SEQ ID NO: 130 - DNA, 21 bp, synthetic construct
  misc_feature 1..21: note = Description of Artificial Sequence: Synthetic oligonucleotide
  source 1..21: mol_type = other DNA
gaagttacctaagttaacaaa

SEQ ID NO: 131 - DNA, 21 bp, synthetic construct
  misc_feature 1..21: note = Description of Artificial Sequence: Synthetic oligonucleotide
  source 1..21: mol_type = other DNA
ggaccactgcagtcaggactc

SEQ ID NO: 132 - DNA, 21 bp, synthetic construct
  misc_feature 1..21: note = Description of Artificial Sequence: Synthetic oligonucleotide
  source 1..21: mol_type = other DNA
ggggtgtcacgtacttataaa

SEQ ID NO: 133 - DNA, 21 bp, synthetic construct
  misc_feature 1..21: note = Description of Artificial Sequence: Synthetic oligonucleotide
  source 1..21: mol_type = other DNA
gttaattgattgcaaatttga

SEQ ID NO: 134 - DNA, 21 bp, synthetic construct
  misc_feature 1..21: note = Description of Artificial Sequence: Synthetic oligonucleotide
  source 1..21: mol_type = other DNA
gaggtaaccaaccaaacaaaa

SEQ ID NO: 135 - DNA, 22 bp, synthetic construct
  misc_feature 1..22: note = Description of Artificial Sequence: Synthetic oligonucleotide
  source 1..22: mol_type = other DNA
gtgtaagatcaaagagacaaga

SEQ ID NO: 136 - DNA, 22 bp, synthetic construct
  misc_feature 1..22: note = Description of Artificial Sequence: Synthetic oligonucleotide
  source 1..22: mol_type = other DNA
ggtccttctccttaggttttta

SEQ ID NO: 137 - DNA, 22 bp, synthetic construct
  misc_feature 1..22: note = Description of Artificial Sequence: Synthetic oligonucleotide
  source 1..22: mol_type = other DNA
gttataatttctagaggaaaat

SEQ ID NO: 138 - DNA, 22 bp, synthetic construct
  misc_feature 1..22: note = Description of Artificial Sequence: Synthetic oligonucleotide
  source 1..22: mol_type = other DNA
gtacgtgacacccctggccaca

SEQ ID NO: 139 - DNA, 22 bp, synthetic construct
  misc_feature 1..22: note = Description of Artificial Sequence: Synthetic oligonucleotide
  source 1..22: mol_type = other DNA
gttttttaaaaatcagatcaac

SEQ ID NO: 140 - DNA, 22 bp, synthetic construct
  misc_feature 1..22: note = Description of Artificial Sequence: Synthetic oligonucleotide
  source 1..22: mol_type = other DNA
gtcctgtcagccaatattagct

SEQ ID NO: 141 - DNA, 22 bp, synthetic construct
  misc_feature 1..22: note = Description of Artificial Sequence: Synthetic oligonucleotide
  source 1..22: mol_type = other DNA
gccaatattagctctgagttat

SEQ ID NO: 142 - DNA, 22 bp, synthetic construct
  misc_feature 1..22: note = Description of Artificial Sequence: Synthetic oligonucleotide
  source 1..22: mol_type = other DNA
gattaacctgaaggtaaaaaga

SEQ ID NO: 143 - DNA, 22 bp, synthetic construct
  misc_feature 1..22: note = Description of Artificial Sequence: Synthetic oligonucleotide
  source 1..22: mol_type = other DNA
tattttatctttagggcttagg

SEQ ID NO: 144 - DNA, 22 bp, synthetic construct
  misc_feature 1..22: note = Description of Artificial Sequence: Synthetic oligonucleotide
  source 1..22: mol_type = other DNA
aaatatattttatctttagggc

SEQ ID NO: 145 - DNA, 22 bp, synthetic construct
  misc_feature 1..22: note = Description of Artificial Sequence: Synthetic oligonucleotide
  source 1..22: mol_type = other DNA
taaatatattttatctttaggg

SEQ ID NO: 146 - DNA, 22 bp, synthetic construct
  misc_feature 1..22: note = Description of Artificial Sequence: Synthetic oligonucleotide
  source 1..22: mol_type = other DNA
ccttttaaatatattttatctt

SEQ ID NO: 147 - DNA, 22 bp, synthetic construct
  misc_feature 1..22: note = Description of Artificial Sequence: Synthetic oligonucleotide
  source 1..22: mol_type = other DNA
accttttaaatatattttatct

SEQ ID NO: 148 - DNA, 22 bp, synthetic construct
  misc_feature 1..22: note = Description of Artificial Sequence: Synthetic oligonucleotide
  source 1..22: mol_type = other DNA
caccttttaaatatattttatc

SEQ ID NO: 149 - DNA, 22 bp, synthetic construct
  misc_feature 1..22: note = Description of Artificial Sequence: Synthetic oligonucleotide
  source 1..22: mol_type = other DNA
gatcacacctaagccctaaaga

SEQ ID NO: 150 - DNA, 22 bp, synthetic construct
  misc_feature 1..22: note = Description of Artificial Sequence: Synthetic oligonucleotide
  source 1..22: mol_type = other DNA
tgatcacacctaagccctaaag

SEQ ID NO: 151 - DNA, 22 bp, synthetic construct
  misc_feature 1..22: note = Description of Artificial Sequence: Synthetic oligonucleotide
  source 1..22: mol_type = other DNA
atgatcacacctaagccctaaa

SEQ ID NO: 152 - DNA, 22 bp, synthetic construct
  misc_feature 1..22: note = Description of Artificial Sequence: Synthetic oligonucleotide
  source 1..22: mol_type = other DNA
gcaatgatcacacctaagccct

SEQ ID NO: 153 - DNA, 22 bp, synthetic construct
  misc_feature 1..22: note = Description of Artificial Sequence: Synthetic oligonucleotide
  source 1..22: mol_type = other DNA
tgcaatgatcacacctaagccc

SEQ ID NO: 154 - DNA, 22 bp, synthetic construct
  misc_feature 1..22: note = Description of Artificial Sequence: Synthetic oligonucleotide
  source 1..22: mol_type = other DNA
ttgcaatgatcacacctaagcc

SEQ ID NO: 155 - DNA, 22 bp, synthetic construct
  misc_feature 1..22: note = Description of Artificial Sequence: Synthetic oligonucleotide
  source 1..22: mol_type = other DNA
attgcaatgatcacacctaagc

SEQ ID NO: 156 - DNA, 22 bp, synthetic construct
  misc_feature 1..22: note = Description of Artificial Sequence: Synthetic oligonucleotide
  source 1..22: mol_type = other DNA
ccttttaaatatattttatctt

SEQ ID NO: 157 - DNA, 21 bp, synthetic construct
  misc_feature 1..21: note = Description of Artificial Sequence: Synthetic oligonucleotide
  source 1..21: mol_type = other DNA
attttatctttagggcttagg

SEQ ID NO: 158 - DNA, 21 bp, synthetic construct
  misc_feature 1..21: note = Description of Artificial Sequence: Synthetic oligonucleotide
  source 1..21: mol_type = other DNA
aatatattttatctttagggc

SEQ ID NO: 159 - DNA, 21 bp, synthetic construct
  misc_feature 1..21: note = Description of Artificial Sequence: Synthetic oligonucleotide
  source 1..21: mol_type = other DNA
aaatatattttatctttaggg

SEQ ID NO: 160 - DNA, 21 bp, synthetic construct
  misc_feature 1..21: note = Description of Artificial Sequence: Synthetic oligonucleotide
  source 1..21: mol_type = other DNA
cttttaaatatattttatctt

SEQ ID NO: 161 - DNA, 21 bp, synthetic construct
  misc_feature 1..21: note = Description of Artificial Sequence: Synthetic oligonucleotide
  source 1..21: mol_type = other DNA
ccttttaaatatattttatct

SEQ ID NO: 162 - DNA, 21 bp, synthetic construct
  misc_feature 1..21: note = Description of Artificial Sequence: Synthetic oligonucleotide
  source 1..21: mol_type = other DNA
accttttaaatatattttatc

SEQ ID NO: 163 - DNA, 21 bp, synthetic construct
  misc_feature 1..21: note = Description of Artificial Sequence: Synthetic oligonucleotide
  source 1..21: mol_type = other DNA
atcacacctaagccctaaaga

SEQ ID NO: 164 - DNA, 21 bp, synthetic construct
  misc_feature 1..21: note = Description of Artificial Sequence: Synthetic oligonucleotide
  source 1..21: mol_type = other DNA
gatcacacctaagccctaaag

SEQ ID NO: 165 - DNA, 21 bp, synthetic construct
  misc_feature 1..21: note = Description of Artificial Sequence: Synthetic oligonucleotide
  source 1..21: mol_type = other DNA
tgatcacacctaagccctaaa

SEQ ID NO: 166 - DNA, 21 bp, synthetic construct
  misc_feature 1..21: note = Description of Artificial Sequence: Synthetic oligonucleotide
  source 1..21: mol_type = other DNA
caatgatcacacctaagccct

SEQ ID NO: 167 - DNA, 21 bp, synthetic construct
  misc_feature 1..21: note = Description of Artificial Sequence: Synthetic oligonucleotide
  source 1..21: mol_type = other DNA
gcaatgatcacacctaagccc

SEQ ID NO: 168 - DNA, 21 bp, synthetic construct
  misc_feature 1..21: note = Description of Artificial Sequence: Synthetic oligonucleotide
  source 1..21: mol_type = other DNA
tgcaatgatcacacctaagcc

SEQ ID NO: 169 - DNA, 21 bp, synthetic construct
  misc_feature 1..21: note = Description of Artificial Sequence: Synthetic oligonucleotide
  source 1..21: mol_type = other DNA
ttgcaatgatcacacctaagc

SEQ ID NO: 170 - DNA, 21 bp, synthetic construct
  misc_feature 1..21: note = Description of Artificial Sequence: Synthetic oligonucleotide
  source 1..21: mol_type = other DNA
cttttaaatatattttatctt

SEQ ID NO: 171 - DNA, 20 bp, synthetic construct
  misc_feature 1..20: note = Description of Artificial Sequence: Synthetic oligonucleotide
  source 1..20: mol_type = other DNA
ttttatctttagggcttagg

SEQ ID NO: 172 - DNA, 20 bp, synthetic construct
  misc_feature 1..20: note = Description of Artificial Sequence: Synthetic oligonucleotide
  source 1..20: mol_type = other DNA
atatattttatctttagggc

SEQ ID NO: 173 - DNA, 20 bp, synthetic construct
  misc_feature 1..20: note = Description of Artificial Sequence: Synthetic oligonucleotide
  source 1..20: mol_type = other DNA
aatatattttatctttaggg

SEQ ID NO: 174 - DNA, 20 bp, synthetic construct
  misc_feature 1..20: note = Description of Artificial Sequence: Synthetic oligonucleotide
  source 1..20: mol_type = other DNA
ttttaaatatattttatctt

SEQ ID NO: 175 - DNA, 20 bp, synthetic construct
  misc_feature 1..20: note = Description of Artificial Sequence: Synthetic oligonucleotide
  source 1..20: mol_type = other DNA
cttttaaatatattttatct

SEQ ID NO: 176 - DNA, 20 bp, synthetic construct
  misc_feature 1..20: note = Description of Artificial Sequence: Synthetic oligonucleotide
  source 1..20: mol_type = other DNA
ccttttaaatatattttatc

SEQ ID NO: 177 - DNA, 20 bp, synthetic construct
  misc_feature 1..20: note = Description of Artificial Sequence: Synthetic oligonucleotide
  source 1..20: mol_type = other DNA
tcacacctaagccctaaaga

SEQ ID NO: 178 - DNA, 20 bp, synthetic construct
  misc_feature 1..20: note = Description of Artificial Sequence: Synthetic oligonucleotide
  source 1..20: mol_type = other DNA
atcacacctaagccctaaag

SEQ ID NO: 179 - DNA, 20 bp, synthetic construct
  misc_feature 1..20: note = Description of Artificial Sequence: Synthetic oligonucleotide
  source 1..20: mol_type = other DNA
gatcacacctaagccctaaa

SEQ ID NO: 180 - DNA, 20 bp, synthetic construct
  misc_feature 1..20: note = Description of Artificial Sequence: Synthetic oligonucleotide
  source 1..20: mol_type = other DNA
aatgatcacacctaagccct

SEQ ID NO: 181 - DNA, 20 bp, synthetic construct
  misc_feature 1..20: note = Description of Artificial Sequence: Synthetic oligonucleotide
  source 1..20: mol_type = other DNA
caatgatcacacctaagccc

SEQ ID NO: 182 - DNA, 20 bp, synthetic construct
  misc_feature 1..20: note = Description of Artificial Sequence: Synthetic oligonucleotide
  source 1..20: mol_type = other DNA
gcaatgatcacacctaagcc

SEQ ID NO: 183 - DNA, 20 bp, synthetic construct
  misc_feature 1..20: note = Description of Artificial Sequence: Synthetic oligonucleotide
  source 1..20: mol_type = other DNA
tgcaatgatcacacctaagc

SEQ ID NO: 184 - DNA, 20 bp, synthetic construct
  misc_feature 1..20: note = Description of Artificial Sequence: Synthetic oligonucleotide
  source 1..20: mol_type = other DNA
ttttaaatatattttatctt

SEQ ID NO: 185 - DNA, 20 bp, synthetic construct
  misc_feature 1..20: note = Description of Artificial Sequence: Synthetic oligonucleotide
  source 1..20: mol_type = other DNA
ttttatctttagggcttagg

SEQ ID NO: 186 - DNA, 20 bp, synthetic construct
  misc_feature 1..20: note = Description of Artificial Sequence: Synthetic oligonucleotide
  source 1..20: mol_type = other DNA
aatatattttatctttaggg

SEQ ID NO: 187 - DNA, 20 bp, synthetic construct
  misc_feature 1..20: note = Description of Artificial Sequence: Synthetic oligonucleotide
  source 1..20: mol_type = other DNA
aaattgcaatgatcacacct

SEQ ID NO: 188 - DNA, 264 bp, synthetic construct
  misc_feature 1..264: note = Description of Artificial Sequence: Synthetic polynucleotide
  source 1..264: mol_type = other DNA
aaggtcgggcaggaagagggcctatttcccatgattccttcatatttgcatatacgatacaaggctgttagagagataattagaattaatttgactgtaaacacaaagatattagtacaaaatacgtgacgtagaaagtaataatttcttgggtagtttgcagttttaaaattatgttttaaaatggactatcatatgcttaccgtaacttgaaagtatttcgatttcttggctttatatatcttgtggaaaggacgaaacacc

SEQ ID NO: 189 - DNA, 40 bp, Mus sp.
  source 1..40: mol_type = genomic DNA
attgggaatgcagtactgctgaacggaggggtggacacgg